European Patent Application EP 4 303 219 A1, published January 10, 2024. Title: 8-(PICOLINAMIDE) SUBSTITUTED COUMARIN COMPOUND, AND PREPARATION METHOD THEREFOR AND USE THEREOF. Applicant: LONGIVITRON (SUZHOU) BIOTECHNOLOGY CO., LTD. The sequence listing filed with the application follows.

SEQUENCE LISTING (2 sequences)

SEQ ID NO: 1 - DNA, 20 bp, Artificial sequence
  primer
taatacgactcactataggg

SEQ ID NO: 2 - DNA, 21 bp, Artificial sequence
  primer
ttcacttctgagttcggcatg